European Patent Application EP 4 324 911 A1, published February 21, 2024. Title: PAENIBACILLUS STRAIN, AND HEMOSTATIC POLYSACCHARIDE PRODUCED BY SAME AND USE THEREOF. Applicant: Nanjing Southern Element Biotechnology Co., Ltd. The sequence listing filed with the application follows.

SEQUENCE LISTING (1 sequence)

SEQ ID NO: 1 - DNA, 1060 bp, Paenibacillus
  source 1..1060: mol_type = genomic DNA; note = 16S rDNA of the selected single colony strain
acaatcttcgacggctggctccttgcggttaccccaccggcttcgggtgttgtaaactctcgtggtgtgacgggcggtgtgtacaagacccgggaacgtattcaccgcggcatgctgatccgcgattactagcaattccgacttcatgcaggcgagttgcagcctgcaatccgaactgagaccgcctttttaggattcgctccagatcgctccttcgcttcccgttgtaacggccattgtagtacgtgtgtagcccaggtcataaggggcatgatgatttgacgtcatccccgccttcctccggtttgtcaccggcagtcattctagagtgcccaccttaaagtgctggcaactaaaatcaagggttgcgctcgttgcgggacttaacccaacatctcacgacacgagctgacgacaaccatgcaccacctgtctcctctgtccccgaagggccgcccctatctctaggggattcaaagggatgtcaagacctggtaaggttcttcgcgttgcttcaaattaaaccacatactccactgcttgtgcgggtccccgtcaattcctttgagtttcactcttgcgagcgtactccccaggcggaatgcttaaggtgttaacttcggcaccaagggtatcgaaacccctaacacctagcattcatcgtttacggcgtgaactaccagggtatctaatcctgtttgctccccacgctttcgcgcctcagcgtcagttacagcccagaaagtcgccttcgccactggtgttcctccacatctctacgcatttcaccgctacacgtggaattccactttcctcttctgcactcaagtcttgcagtttcagatgcgaatcggggttgagccccgagattaaacacctgacttacaaaaccgcctgcgcgcgctttacgcccaaataattccggacaacgcttgccccctacgtattaccgcggctgctggnacgtagttagccggggctttctttctcaggtacgtcatagcagagcagtactctcccactcgttcttccctnnaanagnagctttacgatccggaaa